European Patent Application EP 4 219 764 A1, published August 2, 2023. Title: METHOD FOR DETECTING METABOLIC REPROGRAMING OF CANCER TOWARDS FATTY ACIDS METABOLISM. Applicant: UNIVERSITE DE PARIS INSTITUT NATIONAL DE LA SANTE ET DE LA RECHERCHE MEDICALE. The sequence listing filed with the application follows.

SEQUENCE LISTING (29 sequences)

SEQ ID NO: 1 - protein, 579 aa, Homo Sapiens
MLRSGPASGPSVPTGRAMPSRRVARPPAAPELGALGSPDLSSLSLAVSRSTDELEIIDEYIKENGFGLDGGQPGPGEGLPRLVSRGAASLSTVTLGPVAPPATPPPWGCPLGRLVSPAPGPGPQPHLVITEQPKQRGMRFRYECEGRSAGSILGESSTEASKTLPAIELRDCGGLREVEVTACLVWKDWPHRVHPHSLVGKDCTDGICRVRLRPHVSPRHSFNNLGIQCVRKKEIEAAIERKIQLGIDPYNAGSLKNHQEVDMNVVRICFQASYRDQQGQMRRMDPVLSEPVYDKKSTNTSELRICRINKESGPCTGGEELYLLCDKVQKEDISVVFSRASWEGRADFSQADVHRQIAIVFKTPPYEDLEIVEPVTVNVFLQRLTDGVCSEPLPFTYLPRDHDSYGVDKKRKRGMPDVLGELNSSDPHGIESKRRKKKPAILDHFLPNHGSGPFLPPSALLPDPDFFSGTVSLPGLEPPGGPDLLDDGFAYDPTAPTLFTMLDLLPPAPPHASAVVCSGGAGAVVGETPGPEPLTLDSYQAPGPGDGGTASLVGSNMFPNHYREAAFGGGLLSPGPEAT

SEQ ID NO: 2 - protein, 117 aa, Artificial Sequence
  VH of anti pSer 472 RelB monoclonal antibody
EVQLVETGGGLVQPKGSLKLSCAVSGFTFNTDAMNWVRQAPGKGLEWVARMRSKSNNYATYYADSVKDRCTISRDDSQSMFYLQMNNLKTEDTAMYYCVYGGAMDYWGQGTSVTVSS

SEQ ID NO: 3 - protein, 5 aa, Artificial Sequence
  H-CDR1 of anti pSer 472 RelB monoclonal antibody
TDAMN

SEQ ID NO: 4 - protein, 19 aa, Artificial Sequence
  H-CDR2 of anti pSer 472 RelB monoclonal antibody
RMRSKSNNYATYYADSVKD

SEQ ID NO: 5 - protein, 8 aa, Artificial Sequence
  H-CDR3 of anti pSer 472 RelB monoclonal antibody
VYGGAMDY

SEQ ID NO: 6 - protein, 111 aa, Artificial Sequence
  VL of anti pSer 472 RelB monoclonal antibody
DIVLTQSPASLVVSLGQRATISCRASKSVYTSGYSYMHWFQQKPGQPPKLLIKYASNLQSGVPARFSGSGSGTDFTLNIHPVEAEDTATYYCQHNWEIPLTFGAGTKLELK

SEQ ID NO: 7 - protein, 15 aa, Artificial Sequence
  L-CDR1 of anti pSer 472 RelB monoclonal antibody
RASKSVYTSGYSYMH

SEQ ID NO: 8 - protein, 7 aa, Artificial Sequence
  L-CDR2 of anti pSer 472 RelB monoclonal antibody
YASNLQS

SEQ ID NO: 9 - protein, 9 aa, Artificial Sequence
  L-CDR3 of anti pSer 472 RelB monoclonal antibody
QHNWEIPLT

SEQ ID NO: 10 - DNA, 20 bp, Artificial Sequence
  ABCG1 forward primer
tcagggacctttcctattcg

SEQ ID NO: 11 - DNA, 21 bp, Artificial Sequence
  ABCG1 reverse primer
ttcctttcaggagggtcttgt

SEQ ID NO: 12 - DNA, 19 bp, Artificial Sequence
  ALDH8A1 forward primer
aaccgtcaggtccagcttt

SEQ ID NO: 13 - DNA, 25 bp, Artificial Sequence
  ALDH8A1 reverse primer
cactatagatgctcttctggacaaa

SEQ ID NO: 14 - DNA, 18 bp, Artificial Sequence
  ALPI forward primer
catggaccgcttcccata

SEQ ID NO: 15 - DNA, 19 bp, Artificial Sequence
  ALPI reverse primer
ggcacctgtctgtccacat

SEQ ID NO: 16 - DNA, 20 bp, Artificial Sequence
  CDS2 forward primer
cgattttcccaggatgacag

SEQ ID NO: 17 - DNA, 24 bp, Artificial Sequence
  CDS2 reverse primer
tctacctttgcttctgactctgac

SEQ ID NO: 18 - DNA, 20 bp, Artificial Sequence
  CYP1B1 forward primer
aacgtaccggccactatcac

SEQ ID NO: 19 - DNA, 20 bp, Artificial Sequence
  CYP1B1 reverse primer
ctcgagtctgcacatcagga

SEQ ID NO: 20 - DNA, 18 bp, Artificial Sequence
  ELOVL4 forward primer
catttggcccatggattc

SEQ ID NO: 21 - DNA, 20 bp, Artificial Sequence
  ELOVL4 reverse primer
ccaatggtcacatggaattg

SEQ ID NO: 22 - DNA, 20 bp, Artificial Sequence
  PTGIS forward primer
tgaaaaggccaggatgaaac

SEQ ID NO: 23 - DNA, 22 bp, Artificial Sequence
  PTGIS reverse primer
ggaggttggtatacatggcttc

SEQ ID NO: 24 - DNA, 21 bp, Artificial Sequence
  PRKAR2B forward primer
cccagagcagctacaatcact

SEQ ID NO: 25 - DNA, 21 bp, Artificial Sequence
  PRKAR2B reverse primer
tttttggcattgtttttcaca

SEQ ID NO: 26 - DNA, 23 bp, Artificial Sequence
  UGT2B15 forward primer
gaaaaagaaacagcgtgaaattg

SEQ ID NO: 27 - DNA, 24 bp, Artificial Sequence
  UGT2B15 reverse primer
ttctccaatcctcttattttcctc

SEQ ID NO: 28 - DNA, 19 bp, Artificial Sequence
  HPRT forward primer
ggcgtcgtgattagtgatg

SEQ ID NO: 29 - DNA, 21 bp, Artificial Sequence
  HPRT reverse primer
gcacacagagggctacaatgt